European Patent Specification EP 3 512 538 B1, published December 18, 2024. Title: METHODS FOR ENHANCING LIFESPAN AND/OR TREATING CELLULAR PROLIFERATIVE DISORDERS BY TRANSPLANTATION. Applicant: ACADEMIA SINICA SHEN, CHE-KUN JAMES SHYU, YU-CHIAU HUNG, CHUN-HAO. The sequence listing filed with the application follows.

SEQUENCE LISTING (16 sequences)

SEQ ID NO: 1 - DNA, 20 bp, Artificial sequence
  primer(5'-deletion), synthetic sequence
gcggcgcgataacttcgtat

SEQ ID NO: 2 - DNA, 22 bp, Artificial sequence
  primer(5'-PGK), synthetic sequence
ttgaattctgcttcctgttgga

SEQ ID NO: 3 - DNA, 22 bp, Artificial sequence
  primer(EKLF-F), synthetic sequence
aggcagaagagagagaggaggc

SEQ ID NO: 4 - DNA, 22 bp, Artificial sequence
  primer(3'-deletion), synthetic sequence
cctatttctccaacaggaagca

SEQ ID NO: 5 - DNA, 20 bp, Artificial sequence
  primer(PGK-R), synthetic sequence
ctggccctcaaacaaccctg

SEQ ID NO: 6 - DNA, 22 bp, Artificial sequence
  primer(3'-PGK), synthetic sequence
gttatgcggccctagtgattta

SEQ ID NO: 7 - DNA, 19 bp, artificial sequence
  Eklf Forward sequence, synthetic sequence
ggacacccaggaggacttc

SEQ ID NO: 8 - DNA, 22 bp, Artificial sequence
  Eklf Reverse sequence, synthetic sequence
gggtcctccgatttcagactca

SEQ ID NO: 9 - DNA, 19 bp, Artificial sequence
  Actin Forward sequence, synthetic sequence
atggaggggaatacagccc

SEQ ID NO: 10 - DNA, 19 bp, Artificial sequence
  Actin Reverse sequence, synthetic sequence
ttctttgcagctccttcgt

SEQ ID NO: 11 - DNA, 21 bp, Artificial sequence
  Csf2rb Forward sequence, synthetic sequence
acagagaacctagatcgagcc

SEQ ID NO: 12 - DNA, 21 bp, Artificial sequence
  Csf2rb Reverse sequence, synthetic sequence
gtgtactcttcgctccacttg

SEQ ID NO: 13 - DNA, 20 bp, Artificial sequence
  Stat1 Forward sequence, synthetic sequence
ctgaatatttccctcctggg

SEQ ID NO: 14 - DNA, 21 bp, Artificial sequence
  Stat1 Reverse sequence, synthetic sequence
tcccgtacagatgtccatgat

SEQ ID NO: 15 - DNA, 20 bp, Artificial sequence
  Stat2 Forward sequence, synthetic sequence
gctgtcaaggttctgcaaca

SEQ ID NO: 16 - DNA, 20 bp, Artificial sequence
  Stat2 Reverse sequence, synthetic sequence
cgcttggagaattggaagtt